European Patent Specification EP 4 237 570 B1, published July 15, 2026. Title: Novel process. Applicant: DSM IP Assets B.V. The sequence listing filed with the application follows.

SEQUENCE LISTING (17 sequences)

SEQ ID NO: 1 - protein, 334 aa, Yarrowia lipolytica
MKLSTILFTACATLAAALPSPITPSEAAVLQKRVYTSTETSHIDQESYNFFEKYARLANIGYCVGPGTKIFKPFNCGLQCAHFPNVELIEEFHDPRLIFDVSGYLAVDHASKQIYLVIRGTHSLEDVITDIRIMQAPLTNFDLAANISSTATCDDCLVHNGFIQSYNNTYNQIGPKLDSVIEQYPDYQIAVTGHSLGGAAALLFGINLKVNGHDPLVVTLGQPIVGNAGFANWVDKLFFGQENPDVSKVSKDRKLYRITHRGDIVPQVPFWDGYQHCSGEVFIDWPLIHPPLSNVVMCQGQSNKQCSAGNTLLQQVNVIGNHLQYFVTEGVCGI

SEQ ID NO: 2 - DNA, 1005 bp, Yarrowia lipolytica
atgaagctttccaccatcctcttcacagcctgcgctaccctggctgccgccctcccttcccccatcactccttctgaggccgcagttctccagaagcgagtgtacacctctaccgagacctctcacattgaccaggagtcctacaacttctttgagaagtacgcccgactcgcaaacattggatattgtgttggtcccggcactaagatcttcaagcccttcaactgtggcctgcaatgtgcccacttccccaacgttgagctcatcgaggagttccacgacccccgtctcatctttgatgtttctggttacctcgctgttgatcatgcctccaagcagatctaccttgttattcgaggaacccactctctggaggacgtcataaccgacatccgaatcatgcaggctcctctgacgaactttgatcttgctgctaacatctcttctactgctacttgtgatgactgtcttgtccacaatggcttcatccagtcctacaacaacacctacaatcagatcggccccaagctcgactctgtgattgagcagtatcccgactaccagattgctgtcaccggtcactctctcggaggagctgcagcccttctgttcggaatcaacctcaaggttaacggccacgatcccctcgttgttactcttggtcagcccattgtcggtaacgctggctttgctaactgggtcgataaactcttctttggccaggagaaccccgatgtctccaaggtgtccaaagaccgaaagctctaccgaatcacccaccgaggagatatcgtccctcaagtgcccttctgggacggttaccagcactgctctggtgaggtctttattgactggcccctgatccaccctcctctctccaacgttgtcatgtgccagggccagagcaataaacagtgctctgccggtaacactctgctccagcaggtcaatgtgattggaaaccatctgcagtacttcgtcaccgagggtgtctgtggtatctaa

SEQ ID NO: 3 - protein, 498 aa, Yarrowia lipolytica
MPLELPSLNASIVGNTVQNGAVEQFLNIRYADIPGKFEKPVLKNDWNGAEIDATKVGPVCPQPRTPFNFFSVPDDLWEKVNVDTYQDGLLCDNLIVTRPKGVSANARLPTVVWIHGGSNIEGSIYNLIYEPQFLVAESVRVGKPIVHVCIEYRLGLAGFLTKNGKGNWGTWDQYTGCQWVNRHIQDFGGDPLNVTLTGESAGSVAVHNMLIKDSMNGRKLFRNAVMMSGTLETITPQPPKWHARLEEKVAKVTGKEVADLASLSDKELLDAQIKLNVAVCMTCDDGDFFEPGWKQHLTPDWLDKLIISDCKDEGMLYFLPVNAQDDEELLAKVAKSPVGKEISELYGIKEGGDIKSACLDLKTDATFNYFNHLLFKKMEEARNNGSTSRVYRLAVDEPNPHNPDQRAHHAVDVLYMFNSTKFNEHGDKLSRLFQSHFLRLAYGLEPWDHRNFGVYRNGGYQQLPLSELNKVRPVERYEALSKMDFGQVGRLSNALSRL

SEQ ID NO: 4 - DNA, 1497 bp, Yarrowia lipolytica
atgcctctcgaactcccctcgctcaacgcctcgattgtcggcaacaccgttcagaacggcgctgttgagcagtttctcaacatccgatacgccgacattcctggcaagtttgagaagcccgtgctcaagaacgattggaacggcgcggagatcgacgccaccaaggtcggtcccgtgtgcccccaaccccgcaccccattcaacttcttctccgtgccagacgacctctgggagaaagtcaatgtggacacgtaccaggacggtctgctgtgcgacaacctgattgtgacgcgaccgaagggcgtgtctgccaacgcccggctgcccactgttgtgtggatccacggcggctccaatattgagggcagtatctacaacctcatctatgagccccagttcctggtggcagagtcggtgcgagtaggcaagccgattgtgcacgtgtgtatcgagtaccgactgggtctcgcgggcttcctcaccaagaacggcaagggcaactggggcacgtgggatcagtacacgggctgccagtgggtcaaccgccacattcaggactttggaggcgatcctttgaacgtgacattgaccggtgagtctgccggctctgtagcagtccataacatgctcatcaaggactccatgaacggccgaaagttgttccgaaatgccgtcatgatgagtggcactctcgagaccatcactcctcagcctcccaagtggcatgctcgtttggaggagaaggtggccaaggtcactggcaaggaagtggccgaccttgcttctctgtccgataaggagctgctcgacgcccagatcaagctcaatgtggctgtgtgcatgacttgcgacgacggcgactttttcgagcccggatggaagcagcatctgactcctgactggctcgacaagctcatcatctccgattgcaaggacgagggcatgctgtatttcctgccagtcaacgcgcaggacgacgaggagctgttggcaaaggtggccaagtcgcccgtgggtaaggagatttccgagctttacggcatcaaggagggtggcgatatcaagtctgcgtgtctcgatctcaagactgacgccaccttcaattactttaaccatctgctgttcaagaagatggaggaggcccgaaacaacggctccacttctcgagtttaccgtctggccgtcgatgagcccaacccccacaaccccgaccagcgggcccaccacgccgtcgacgtgctgtacatgttcaactcgaccaagttcaacgagcacggcgacaagctgtctcggctgttccagagccactttttgcggctggcgtatggcctggagccctgggaccatcgaaactttggagtgtacagaaacggcggctaccagcagctgccgctgagtgagttgaacaaggtccgacccgtcgagcggtacgaggcgctgtccaagatggactttggccaggttgggcgtttgtccaatgcgctttcgcgcctatga

SEQ ID NO: 5 - protein, 371 aa, Yarrowia lipolytica
MVSLSARIKDFFSVLLLGAATITPSTQTAGVSQGFYDFARDFAHLSNIAYCVNAPITPLNPDFTCGNSCKHFPEIELVKTFGGNFFKTSITGYLAVDHVKKEKYVVFRGTFSLADAITDMQFQLSPFLVDVPALNTFSANDTTAEAQTHCEGCKIHDGFSKAFTETWGNIGEDLQKHLDANPDYQLYVTGHSLGAAMALLGATSIKLKGYDPILINYGQPRVGNKPFAEFINKLWFGEGNGLEITPERKLYRMTHWNDIFVGLPNWEGYTHSNGEVYINNRFINPPLKDVISCAGGENSKCYRSSFSLLSQINLLQNHLAYIDYIGYCALNIGRRELADQEHYTGPYYYGHRSEEDFKKLGLELSTPQVEN

SEQ ID NO: 6 - DNA, 1116 bp, Yarrowia lipolytica
atggtatccctctctgctcgaatcaaagactttttttcggtcctcctcctcggagctgcaaccatcactccctccacacagaccgcaggcgtgtctcaagggttctatgattttgctcgggactttgcccatctgtccaacattgcctactgtgtcaatgctcccatcactccactgaacccggacttcacctgtggcaactcgtgcaagcactttccggaaattgagcttgtgaagacatttggaggcaacttcttcaagacctccattacgggctacctggctgtcgatcatgtcaagaaggagaagtacgttgtcttccgaggaaccttttcgctggcagacgcgatcacggacatgcagttccagctgtctcctttcctggtcgatgtgcctgccctgaacactttctcagctaatgacaccaccgcagaggcccagacgcactgtgagggctgcaaaattcacgacggcttctccaaggcctttaccgagacctggggtaacattggtgaggatctgcagaaacacctggacgctaacccggactaccagctgtacgtgactggccattctctgggagctgctatggcccttcttggagctacttccatcaagctcaagggctacgatcccattctcatcaactacggacagccccgagtcggaaacaagcccttcgctgagttcattaacaagttgtggtttggagaaggcaacggtctggaaatcacccccgagagaaagctgtaccgaatgacccactggaacgacatctttgttggcctgcccaactgggagggatacacccactctaacggtgaagtatacatcaacaaccggttcatcaaccctcctctcaaggatgtcatctcttgtgctggaggcgaaaactcgaagtgctaccgatcctcgttcagcctgctgtcccagatcaatctgctccaaaaccacctggcttacattgattacattggatactgcgctctgaacattggtcgacgagagcttgccgatcaggaacattacactggtccttattactatggtcatcgatctgaggaggactttaagaagttgggcttggagctatccaccccacaagttgagaactga

SEQ ID NO: 7 - protein, 406 aa, Yarrowia lipolytica
MAGFNFTFGQVISYLASMLYGQVDATSSSTRIQATQDLYDFTAKFSRLSNIAYCINAPFTPLRTDFTCGESCRYFPDLQLDSVFGGNFSSASTTGYIAYDHKKKEKYIVFRGTFSIPDIITDIQFQTAPWLTSLPTHLIPTKEDFEHKQAILKHYAAENKGLSNLEERQDVVHEDPSLVPKKMDKCENCQIHDGFAKGFNETIEHAGPQIEKFLGNNTDYKMFVVGHSLGAAQAQLFATQFKLLGFDPYMINFGQPRLGNPEFAAYINQLWFNDTGLVVNDARRFYRVTHWNDIVVGVPDWLNYTHSIGEVFIDEESVYPKLDKVVVCEGGENPLCHRGTFNLWSRINFLQNHLAYIFYIGLCAFNIGRRDVLNMPQYQGNFSYQHNIDPNYNYDTKVPTRISKSN

SEQ ID NO: 8 - DNA, 1221 bp, Yarrowia lipolytica
atggcagggttcaacttcactttcgggcaggtgatttcgtacctggcttccatgctctatggacaggtggatgccacttcatcctccactcgaatccaggccacccaggatctgtacgacttcacagccaagttttcgcgactctcaaacatcgcgtactgcatcaatgcccccttcacgcctctcagaacggacttcacctgcggagaaagctgtcggtacttccccgacctccagctggactcagtgtttggtggtaacttctcctcagcctccactaccggctacattgcatacgaccacaagaagaaggaaaagtacattgtgtttcgaggaactttcagtatccctgatatcatcacagacattcaatttcagactgccccttggttgacctctctgcccacgcatctgatccctaccaaggaggactttgaacacaagcaggccatcctgaagcactacgctgccgaaaacaagggtctcagcaacctggaagagcgacaggatgttgtgcatgaagaccctagcctggttcccaagaaaatggacaagtgcgagaactgccagatccatgacggattcgccaagggcttcaacgagactatcgagcatgccggaccccagattgaaaagttcctgggcaataacaccgactacaagatgtttgttgttggccactctctaggagctgctcaggcccagctgtttgctacacagttcaaactgctgggatttgacccttacatgatcaactttggacagcctcgacttggaaaccctgagttcgccgcctacatcaaccagctgtggttcaacgatactggtctggttgtcaatgatgcccgacgattctaccgagtgactcactggaacgatatcgtcgtgggagtgcccgactggctcaattacacccactctatcggagaggtgttcatagacgaggagagcgtttaccccaagctggacaaggtggtggtgtgcgagggaggagagaaccccctgtgccaccgaggaactttcaacctgtggtcacgaatcaacttcctgcagaaccatttggcttatatcttctacattggtctgtgtgctttcaacattggccgaagagacgtgctcaacatgccacaataccagggcaacttctcgtaccagcacaacatcgaccccaactacaattacgataccaaggttcccacccggatcagtaaatcaaactaa

SEQ ID NO: 9 - DNA, 11606 bp, Artificial Sequence
  expression plasmid
cgcgtggatcgccggtgcgttgacgttggtgacctccagccagaggtgcccggcgccccgctcgccggcgaactccgtcgcgagccccatcaacgcgcgcccgaccccgtgcccccggtgctccggggcgacctcgatgtcctcgacggtcagccggcggttccacgccgagtacgagatgaccacgaagcccgccaggtcgccgtcgtccccgtacgcgacgaacgtccgggagtccgggtcgccgtcctccccgtcgtccgattcgtcgtccgattcgtcgtcggggaacaccttggtcaggggcgggtccaccggcacctcccgcagggtgaagccgtccccggtggcggtgacgcggaagacggtgtcggtggtgaaggacccatccagtgcctcgatggcctcggcgtcccccgggacactggtgcggtaccggtaagccgtgtcgtcaagagtggtcatttttgtgtctaggtgtttgtgtttggactgcgatcagtgaagaaaagaagaggaaaaattgtgcaagaaattttgctttcaagacttggctgatgcagcagggtaactctgggacacagacctatgtttgtggttaaactcaatgcacgtggtacgtgcgtggagcgcttacccatccaagggtgtggacatggaaccgacggtccgtggagttgtgtaatgtcattttggcgactcttgaagcaaggctataaaaaaattgtgtggcttgagtcttatcgagctcggtcactacaagagttaatcttcctgtctcaggcagacaggtcaggcagggttacttttgggtgtgctgtaactcactgtatggccgttagtgcgcatagacgttgtacatactggaccgaattgtagcgtgctcaatagggccaataaagctattgtagggatccgaattttcagaacctaatttatctgttacccggcctgtggctcgcacagcttaaaaatggtcaaactttccccttcttgtctttttttcctcacattcatcaggttcttgtcttgatctttcaagtgagtattaattaccgaccttggttcttcattgggagagcattggaagccgtggtgcagcaaccacaaaacggttcttccccttcgataccttcttgcctgcctttcaatacaagtcggctcgattagcggtggtcgcccccgccagcggagaacatggaactaacccagaatgagagctaagtggagaaagaagagagtcagacgactcaagcgaaagcgccgcaaggtccgagctcgatccaaataagcggtttttaacggagatttaacactaaatcgaagaacttttcccgtttcatttgcgaatgagctcgttaacaaaatcccccagtttttttatccagctgtaaggattgacattagtaatgaattattgtttggtatatttaaatctgtagttcctttctgtccgtgtcggcaactgtcgtactcgtgatttacttgtattgacgaatacttactgtagcgcactctgctgctactggtcgtaaggatgtgctatttcggtgtatggtgggttttttgggggtcggaaccgaagactgttacacgggcacggctcgttgtgtacacgcacagagctcttgcgagtcatgttgtagctagctcgtcgtgttcaggaactgttcgatggttcggagagagtcgccgcccagaacatacgcgcaccgatgtcagcagacagccttattacaagtatattcaagcaagtatatccgtagggtgcgggtgatttggatctaaggttcgtactcaacactcacgagcagcttgcctatgttacatccttttatcagacataacataattggagtttacttacacacggggtgtacctgtatgagcaccacctacaattgtagcactggtacttgtacaaagaatttattcgtacgaatcacagggacggccgccctcaccgaaccagcgaatacctcagcggtcccctgcagtgactcaacaaagcgatatgaacatcttgcgatggtatcctgctgatagtttttactgtacaaacacctgtgtagctccttctagcatttttaagttattcacacctcaaggggagggataaattaaataaattccaaaagcgaagatcgagaaactaaattaaaattccaaaaacgaagttggaacacaaccccccgaaaaaaaacaacaaacaaaaaacccaacaaaataaacaaaaacaaaataaatatataactaccagtatctgactaaaagttcaaatactcgtacttacaacaaatagaaatgagccggccaaaattctgcagaaaaaaatttcaaacaagtactggtataattaaattaaaaaacacatcaaagtatcataacgttagttattttattttatttaataaaagaaaacaacaagatgggctcaaaactttcaacttatacgatacataccaaataacaatttagtatttatctaagtgcttttcgtagataatggaatacaaatggatatccagagtatacacatggatagtatacactgacacgacaattctgtatctctttatgttaactactgtgaggcattaaatagagcttgatatataaaatgttacatttcacagtctgaacttttgcagattacctaatttggtaagatattaattatgaactgaaagttgatggcatccctaaatttgatgaaagatgaaattgtaaatgaggtggtaaaagagctacagtcgttttgttttgagataccatcatctctaacgaaatatctattaaaaatctcagtgtgatcatgagtcattgccatcctggaaaatgtcatcatggctgatatttctaactgtttacttgagataaatatatatttacaagaacttcccttgaaattaatttagatataaaatgtttgcgggcaagttactacgaggaataaattatatctagaggttccgcttcctcgctcactgactcgctgcgctcggtcgttcggctgcggcgagcggtatcagctcactcaaaggcggtaatacggttatccacagaatcaggggataacgcaggaaagaacatgtgagcaaaaggccagcaaaaggccaggaaccgtaaaaaggccgcgttgctggcgtttttccataggctccgcccccctgacgagcatcacaaaaatcgacgctcaagtcagaggtggcgaaacccgacaggactataaagataccaggcgtttccccctggaagctccctcgtgcgctctcctgttccgaccctgccgcttaccggatacctgtccgcctttctcccttcgggaagcgtggcgctttctcatagctcacgctgtaggtatctcagttcggtgtaggtcgttcgctccaagctgggctgtgtgcacgaaccccccgttcagcccgaccgctgcgccttatccggtaactatcgtcttgagtccaacccggtaagacacgacttatcgccactggcagcagccactggtaacaggattagcagagcgaggtatgtaggcggtgctacagagttcttgaagtggtggcctaactacggctacactagaaggacagtatttggtatctgcgctctgctgaagccagttaccttcggaaaaagagttggtagctcttgatccggcaaacaaaccaccgctggtagcggtggtttttttgtttgcaagcagcagattacgcgcagaaaaaaaggatctcaagaagatcctttgatcttttctacggggtctgacgctcagtggaacgaaaactcacgttaagggattttggtcatgagattatcaaaaaggatcttcacctagatccttttaaattaaaaatgaagttttaaatcaatctaaagtatatatgagtaaacttggtctgacagttaccaatgcttaatcagtgaggcacctatctcagcgatctgtctatttcgttcatccatagttgcctgactccccgtcgtgtagataactacgatacgggagggcttaccatctggccccagtgctgcaatgataccgcgagacccacgctcaccggctccagatttatcagcaataaaccagccagccggaagggccgagcgcagaagtggtcctgcaactttatccgcctccatccagtctattaattgttgccgggaagctagagtaagtagttcgccagttaatagtttgcgcaacgttgttgccattgctgcaggcatcgtggtgtcacgctcgtcgtttggtatggcttcattcagctccggttcccaacgatcaaggcgagttacatgatcccccatgttgtgcaaaaaagcggttagctccttcggtcctccgatcgttgtcagaagtaagttggccgcagtgttatcactcatggttatggcagcactgcataattctcttactgtcatgccatccgtaagatgcttttctgtgactggtgagtactcaaccaagtcattctgagaatagtgtatgcggcgaccgagttgctcttgcccggcgtcaacacgggataataccgcgccacatagcagaactttaaaagtgctcatcattggaaaacgttcttcggggcgaaaactctcaaggatcttaccgctgttgagatccagttcgatgtaacccactcgtgcacccaactgatcttcagcatcttttactttcaccagcgtttctgggtgagcaaaaacaggaaggcaaaatgccgcaaaaaagggaataagggcgacacggaaatgttgaatactcatactcttcctttttcaatattattgaagcatttatcagggttattgtctcatgagcggatacatatttgaatgtatttagaaaaataaacaaataggggttccgcgcacatttccccgaaaagtgccacctgacgtctaagaaaccattattatcatgacattaacctataaaaataggcgtatcacgaggccctttcgtctggcctaggaagcgacttccaatcgctttgcatatccagtaccacacccacaggcgtttgtgctactctactgatagcaatagatgcgtcataattggttggcccgctgagcctccacaggatactattgcacataccctggtcatgtgcagatcagctcatttgtggagactctggagtaacttagacgacgcctggttcaattgccgcaatgtgcgcccacgcagataatgtattgaggggtggagcgcctcttggggacttgctgtacttgtacgggatattaaacgcactcagcaagaccatgacgtaaaacacacctactgtacgatacgtactgtaggtattgtactcgtacccggtactacaaatagtacgatactatacggagtgtatttgtaccttgatatacgactggcggagtgaagagaaggagttgaacaagaccagatggggatatcagccccagtgctttgtattacaagtacgagtacttaatagatactgtaaggctattgatacggatggcagtaagtcattgagtaagcaattgtggcccagcatctcccctacgtacttgtaccataccccatggagacaccaatggtctttcacgcacactgtcgtgtgctgtatcgcagaatcgggtgtccaaccaaatgccgttacccccacgtcacagccgatagacagatacaccatcaataccagcaggttgtatcatgcggttggctgaaggtaagctgattggtctaaaaactgtagctgtcctaattcaacgagcgctatttggggccaaccacctcggccaagcggcctttaatctgcgtgccccagaggcgtctaatgaggctctggccgccactgtaggagtgtttctctgtgcgcacacgcagttttgagtttgggcgactttccctttttcccaattgcgtacacacacagctccgagctaagcgctgtccttgaaccttctccctcttttccctctttttctcttccccttcccctcctccacattaaggccaaatcctgaattgcaccaactagtacaacgacaacaatggacaagaagtactccatcggtttggacattggtactaactctgtcggctgggccgtcatcaccgacgagtacaaggttccctccaagaagttcaaggtccttggcaacaccgaccgacactctatcaagaagaacctgatcggtgctctgctgttcgactctggcgagactgccgaggccacccgactgaagcgaaccgctcgacgccgatacacccgacgaaagaaccgaatctgttacctccaggagatcttcagcaacgagatggctaaggtcgacgactccttcttccaccgactcgaggagtctttcctggtcgaagaggataagaagcacgagcgacaccccatcttcggcaacattgttgatgaggttgcctaccatgagaagtaccccaccatctaccacctccgaaagaagctcgtcgactccactgacaaggctgacctccgactcatctaccttgctctcgcccacatgatcaagttccgaggtcacttcctcattgagggtgatctcaaccccgacaactccgacgttgacaagctgttcatccagctcgtccagacctacaaccagctctttgaggagaaccctatcaacgcttctggtgttgacgccaaggccattctctccgcccgactctctaagtcccgacgactcgagaacctcattgcccagctgcccggcgagaagaagaacggcctcttcggtaacctgattgctctctctcttggtctgacccccaacttcaagtccaactttgacctcgccgaggacgccaagctccagctgtccaaggacacctacgatgacgatctggacaacctcctggcccagatcggtgaccagtacgccgatctcttccttgccgccaagaacctctccgacgccatcctgctctccgacatcctccgagtcaacaccgagattaccaaggctcctctgtctgcctctatgatcaagcgatacgacgagcaccaccaggatctcactcttctcaaggctctcgtccgacagcagctccccgagaagtacaaggagattttctttgaccagtccaagaacggttacgctggctacattgacggtggtgcttcccaggaagagttttacaagttcatcaagcctattctggagaagatggacggtaccgaggagctgctcgtcaagctcaaccgagaggacctccttcgaaagcagcgaaccttcgataacggctccatcccccaccagatccacctgggtgagctccacgccattctccgaagacaagaggacttctaccccttcctaaaggataaccgagagaagatcgagaagattctcaccttccgaatcccctactacgtcggtcccctcgctcgaggtaactcccgatttgcttggatgacccgaaagtccgaggagactatcaccccctggaactttgaagaggtagtcgacaagggtgcctccgcccagtctttcattgagcggatgaccaacttcgataagaacctccccaacgagaaggtccttcccaagcactctctcctctacgagtacttcaccgtctacaacgagctgaccaaggtcaagtacgttaccgagggcatgcgaaagcccgctttcctctctggtgagcagaagaaggccattgtcgacctcctgttcaagactaaccgaaaagtcaccgtcaagcagctcaaggaagactacttcaagaagattgagtgcttcgactccgtcgagatttccggtgtcgaggaccgattcaacgcctccctcggcacctaccacgatcttctgaagatcatcaaggacaaggactttcttgataacgaggagaacgaggacattctcgaggacatcgtcctcaccctcacccttttcgaggatcgagagatgatcgaggagcgactcaagacctacgcccatctcttcgacgacaaggtcatgaagcaactcaagcgacgacgatacactggctggggccgactttcccgaaagctcatcaacggcatccgagacaagcagtctggcaagaccatcctggacttcctgaagtccgacggtttcgccaaccgaaacttcatgcagctcatccacgacgactctcttaccttcaaagaggatatccagaaggcccaggtttctggccagggcgactccctccacgagcacattgccaacctcgccggatcccccgccatcaaaaagggtatcctccagaccgtcaaggttgtcgacgaactcgtgaaggtcatgggccgacacaagcccgagaacatcgttatcgagatggcccgagagaaccagaccacccagaagggtcagaagaactcccgagagcgaatgaagcgaatcgaagagggtatcaaggagctcggttcccagattctcaaggagcaccccgtcgagaacacccagctccagaacgagaaactctacctgtactacctccagaatggccgagacatgtacgttgaccaggagctcgacatcaaccgactctccgactacgacgtcgaccacattgttcctcagtccttcctcaaggacgactccatcgacaacaaggttctgacccgatctgacaagaaccgaggtaagtccgacaacgttccctccgaagaggtcgttaagaagatgaagaactactggcgacagcttctcaacgccaaactgatcacccagcgaaagtttgacaacctcaccaaggccgagcgaggtggtctgtccgagctggacaaggccggcttcattaagcgacagctggtcgagactcgacagatcaccaagcacgtcgcccagatcctcgactcccgaatgaacaccaagtacgacgagaacgacaagctcatccgggaggtcaaggtcatcaccctgaagtctaagcttgtctccgacttccgaaaggacttccagttctacaaggtccgagagatcaacaactaccaccacgcccacgacgcctacctcaacgccgttgttggtaccgccctcatcaagaagtatcccaagctcgagtccgagttcgtttacggcgactacaaggtttacgatgtccgaaagatgattgccaagtccgagcaggagatcggtaaggccaccgccaagtactttttctactccaacatcatgaatttcttcaagaccgagatcactctcgccaacggtgagattcgaaagcgacccctgattgagactaatggtgagactggtgagatcgtctgggataagggccgagacttcgccaccgtccgaaaggtcctgtccatgccccaggtcaacattgtcaagaagaccgaggtccagaccggtggcttctccaaggagtccattctccccaagcgaaactccgacaaactcatcgcccgtaagaaggactgggatccgaagaagtacggtggtttcgattctcccaccgttgcctactccgtcctcgttgttgctaaagtcgagaagggtaagtctaagaaactcaagtccgtgaaggagctactcggtatcaccatcatggagcgatcttcttttgagaagaaccccattgacttcctcgaggccaagggttacaaagaggtcaagaaggacctgattatcaagctgcccaagtactccctctttgagctcgagaacggccgaaagcgaatgctggcttccgctggtgagctgcagaagggcaacgagctcgctctgccctccaagtacgtcaacttcctctacctggcctcccactacgagaagctcaagggctcccccgaggacaacgagcagaagcagctgttcgttgagcagcacaagcactacctcgacgagatcatcgagcagatctccgagttctccaagcgagtcatcctcgctgacgccaaccttgataaggttctctctgcttacaacaagcaccgggacaagcccatccgagagcaggccgagaatatcatccacctcttcactctcaccaacctcggcgctcctgctgccttcaagtacttcgacaccaccattgaccgaaagaggtacacctccaccaaggaagtcctcgacgccaccctgatccaccagtccatcaccggcctctacgaaacccgaatcgacctctcccagctcggcggtgactctcgagccgaccccaagaagaagcgaaaagtctaaatatccgaagatcaagagcgaagcaagttgtaagtccaggacatgtttcccgcccacgcgagtgatttataacacctctcttttttgacacccgctcgccttgaaattcatgtcacataaattatagtcaacgacgtttgaataacttgtcttgtagttcgatgatgatcatatgattacattaatagtaattactgtatttgatatatatactaattacaatagtacatattagaacatacaatagttagtgccgtgaagtggcttaaaataccgcgagtcgattacgtaatattattacctcttgcccatcgaacgtacaagtactcctctgttctctccttcctttgctttgtgcacgaagaactgcggtcaggtgacacaactttttccatctcagggtgtgtcgcgtgtgcttcatccaaactttagttggggttcgggttcgcgcgagatgatcacgtgccctgatttggtgtcgtcccccgtcgcgctgcgcacgtgatttatttatttccggtggctgctgtctacgcggggccttctctgcccttctgtttcaaccttcgggcggttctcgtaaccagcagtagcaatccatttcgaaactcaaagagctaaaaacgttaaacctcagcagtcgctcgacgaatgggctgcggttgggaagcccacgaggcctatagccagagcctcgagttgacaggagcccagacgccttttccaacggcaacttttatataaaatggcaatgtattcatgcaattgcggccgtgtcaggttggagacactggaccacactctccattgcttcctgaggagatggatcattgctagtgcatctacgcgcagcaatcccgcaagctcgacaaccgtagatgggctttggtgggccaatcaattacgcaacccgcacgttaaattgtatgaggaaggaaggccacggtacaaagtgggtggtcttcacccagtggttgttggtggcgtcatgcagaccatggccgccagtgtgctggaattgaatatttaccgttcgtataatgtatgctatacgaagttataccggtctcgtagtgttcacgttcagttcacggtgagcttaaaactatcttcaagaagagatttgagacctgatttatacttgcagcaatgtttacttcttatcgcgatacacgaatgtgatacggatcaaagtaagcaggactacgataagataacgaatgcggtgcagtccatgtcgattaggtatagatacatttattttgtgttatgttacattttggggggatactgtcctacttgtagtacctacttgtagtggcgcgttaggggcagggcatgctcatgtagagcgcctgccgctcgccgtccgaggcggtgccgtcgtacagggcggtgtccaggccgcagagggtgaaccccatccgccggta

SEQ ID NO: 10 - DNA, 14006 bp, Artificial Sequence
  expression plasmid
gcggagcctaggccggccagcgtggcgcgtggccatattggccagcagcttactacagctcagccaaagtggatcatgatggacggaaatatcggactggaggccaaaaaggaggtgctcaaatacgcacgggacaagtctgcacaggtggcattcgaacccacgtctgtccccaaagccgctgctctttccgagctcaatctgcccgtttaccccaacaactccattgccttagccacccccaacactgcagagctcgaggccatgttcgaggcattccacgagaagggccgatttgacgttgacgactggtttccagtcatagacggtcttgctctcggagctgactttagaaacggagccaccatgttgtcgcaccaacatcgtggactcaaagctattctcgaacaaggaactctggcccaggcaatccacatgctaccatacatcccaactttgatcatcaagggcggagccaacggcgtcgtcgtcttccaactcattgatgatatcgagtctgccattcattcacagcgttctgcttccaataaaacgcctggcctgttccagaagggcaacgctgcgagtggaaacaccaaggtcggcgtctacatgcagtactttgagcccgaagaagtgggcagtcagtcgattgtaagcgtgactggagctggagacactctgtttggaaccctggccatggagattgtcaaggacgagtcctggttgaacgatatgggagacaagaagagtgcagttgtttctcgagccatgaacaatgctgtgaagactattcagagtaaggacgctgtctgcaagagcatcctttaagtgatttgccatgctttctcttcttccacgatgtaaatacttattttacacactactgtgcagtagcaaatacagaacaagagttgtcgcctattgacagtacagtacgagtagtgtatgtacagtagttatacaatatctatgtgaaattcgtcggcagctttcggctgatgaactacgagttcttcgtaataaatcatcaacgtaataagcttggtaccagagacgggttggcggcgtatttgtgtcccaaaaaacagccccaattgccccaattgaccccaaattgacccagtagcgggcccaaccccggcgagagcccccttcaccccacatatcaaacctcccccggttcccacacttgccgttaagggcgtagggtactgcagtctggaatctacgcttgttcagactttgtactagtttctttgtctggccatccgggtaacccatgccggacgcaaaatagactactgaaaatttttttgctttgtggttgggactttagccaagggtataaaagaccaccgtccccgaattacctttcctcttcttttctctctctccttgtcaactcacacccgaaatcgttaagcatttccttctgagtataagaatcattcgctagccacaaaaatgggtgatctcgatgcccgaggaacctctgctcaccccgagctctctgagcgaccttctattatgccttctatgtctgatattcaggacccttctggtgatgacaaggctactccccgaggatctgctgctggtctgccccagcttgagcttgctggacacgcccgacgacttggccaccttgagaacttctttgctgtccaggctcgacagcagatttactcttcttttgctgttttttgtgagtttgacactgcttgttctctcgctcagcttgcttctgctgtgcgaaacgtttgtctttctaacccccttctccttcacactgttgagcctaagcaccctgacatcgctggattctaccactctgacgagtacctttcccgaccttggcctcagcacgattacatgcgagttcttcgagaggttcacgtcgctgacgttgttatgaacggacagaaggagcacgctcacgttgttcgagatgctgttgacgtttttcaggctcacggaaaccaggttacttctgagctccttgagcttatgactcagattgagattcctcacgcttctcagactcgaccctcttggcgacttctctgttttccccacggagaggctaaccgatggcgaacctttgcttttgtttctaaccactgttcttctgatggtctttctggtcttaacttctttcgagatctccagaaggagcttgctcacggccccacctctggtgctcctggtgcccccggagcttccggagttattttcgattacgctcaggacgctgctaccctgcccaagctgccccctcccattgatcagaagctcgattaccgaccttctaagaaggctcttctcggccttctcgctggcaagttcgttcgagagaagctcggttacgtttctgctgctcctcccactacccctacctctgaccttgctcaccctgagggtcaccagtactactgttaccttgttaacgttcccacttcttctgttgcccacattaagactcaggtgcgagagaacgttcctcacaagtgtactctcactccctttctccaggcttgttggcttgtttctctgttcaagtacggtcgagttttttctggttcttggcttgagcgatacaccgatgttcttgttgctatgaacactcgacagcttctccccgaggaccttgagcttcagcgacagtaccgatacggttctaacattggagctgttcgatacaactaccctattgctccccttgacgttcgagataacgatcagaagttctggtcccttgttgagtcttaccgacttgccctttctgatgcccgagataagaacgattacctttacgctcttggtgctcttatgctccctgagatttacgagaagaagaacgttgatgctgttgttaacgataccattcttaaccagcgacgacagggaacccttctttctaacgttggttacgttcgagatgagcagcccactgcttttgctattaagaaccacgttttttctcagggagttggagctaaccgaaacgcttttgttcttaacatttgtgctaccgatcagggtggtcttaacatcgctatttctattgctaagggaacccttgcttctcgacaggagggacaggagctttgtgatatttttaagtctactctccttcgattttaaacgcgtctatccgaagatcaagagcgaagcaagttgtaagtccaggacatgtttcccgcccacgcgagtgatttataacacctctcttttttgacacccgctcgccttgaaattcatgtcacataaattatagtcaacgacgtttgaataacttgtcttgtagttcgatgatgatcatatgattacattaatagtaattactgtatctgtacctgctgtggaccacgcacggcggaacgtaccgtacaaatattttcttgctcacatgactctctctcggccgcgcacgccggtggcaaattgctcttgcattggctctgtctctagacgtccaaaccgtccaaagtggcagggtgacgtgatgcgacgcacgaaggagatggcccggtggcgaggaaccggacacggcgagccggcgggaaaaaaggcggaaaacgaaaagcgaagggcacaatctgacggtgcggctgccaccaacccaaggaggctattttgggtcgctttccatttcacattcgccctcaatggccactttgcggtggtgaacatggtttctgaaacaaccccccagaattagagtatattgatgtgtttaagattgggttgctatttggccattgtgggggagggtagcgacgtggaggacattccagggcgaattgagcctagaaagtggtaccattccaaccgtctcagtcgtccgaattgatcgctataactatcacctctctcacatgtctacttccccaaccaacatccccaacctcccccacactaaagttcacgccaataatgtaggcactctttctgggtgtgggacagcagagcaatacggaggggagattacacaacgagccacaattggggagatggtagccatctcactcgacccgtcgacttttggcaacgctcaattacccaccaaatttgggctggagttgaggggaccgtgttccagcgctgtaggaccagcaacacacacggtatcaacagcaaccaacgcccccgctaatgcacccagtactgcgcaggtgtgggccaggtgcgttccagatgcgagttggcgaaccctaagccgacagtgtactttttgggacgggcagtagcaatcgtgggcgtagaccccggtgtatataaaggggtggagaggacggattattagcaccaacacacacacttatactacatgctagccacaaaaatgctctctttcttctggcgaaacggtatcgagactcccgagcccctcaaggctgacgtttccggctctatccctccctggcttcagggaacccttctccgaaacggtcctggtctgttctccgttggcaacacttcctacaagcactggttcgatggtatggctctcattcactccttcacctttaaggatggtgaggttttttaccgatctaagtacctgaagtctgagacttacaagaagaacatcgctgccgaccgaatcgttgtgtctgagttcggaaccatggtgtaccccgatccctgcaagaacattttctcccgagccttctcttacatgatgaacgccattcctgactttaccgataacaacctcattaacatcattaagtacggtgaggattactacgcctcctctgaggtcaactacatcaaccagattgaccccctgacccttgagactctcggacgaactaactaccgaaaccacattgccatcaaccttgccactgctcaccctcactacgacgaggagggtaacacttacaacatgggcactgctattatgaacctcggtcgacccaagtacgtgattttcaaggtgcccgccaacacctctgataaggagaacaagaagcctgccctctctgaggtggagcaggtttgctccattcccatccgaccctccctttacccttcttacttccactcttttggcatgactgagaactacatcatcttcgttgagcaggccttcaagctggacatcgtcaagctggctactgcttacttccgagatattaactggggatcttgccttaagttcgaccaggatgacattaacgtgttccacctggtcaacaagaagactggtaaggctgtgtccgtgaagtactacactgacccctttgttaccttccaccacatcaacgcttacgaggacgatggccacgtcgtcttcgatctcattacttacaaggactctaagctgtacgatatgttctacattcagaacatgaagcaggacgtcaagcgatttattgagactaacaaggacttcgctcagcccgtgtgccagcgatttgtccttcccgtcaacgttgataaggagactcctcaggacatcaaccttgtcaagctgcaggacaccactgccactgctgtcctgaaggaggacggctctgtctactgcacccctgacatcatttttaagggtcttgagctccctgctatcaactacaagtttaactctaagaagaaccgatacttctacggcacccgagtggagtggtccccttaccctaacaaggtcgctaaggtggacgttgttactcgaacccacaagatttggactgaggaggagtgttacccttctgagcctgtctttattgcctcccctgacgccgttgatgaggatgacggtgtgattctttcttctgtggtttctttcaacccccagcgaccccctttcctggttgtcctcgatgctaagtccttcaaggagattgctcgagctaccatcgatgcctctattcacatggaccttcacggccttttcatccacgacaagtctacctaagttttttgatcaatgatccaatggctttcacatacccccccacgcctataattaaaacacagagaaatataatctaacttaataaatattacggagaatctttcgagtgttcagcagaaatatagccattgtaacaaaagccggctatcgaccgctttatcgaagaatatttcccgccccccagtggccaaacgatatcggtcagaaggggcagctctaaacgaagaactgcggtcaggtgacacaactttttccatctcagggtgtgtcgcgtgtgcttcatccaaactttagttggggttcgggttcgcgcgagatgatcacgtgccctgatttggtgtcgtcccccgtcgcgctgcgcacgtgatttatttatttccggtggctgctgtctacgcggggccttctctgcccttctgtttcaaccttcgggcggttctcgtaaccagcagtagcaatccatttcgaaactcaaagagctaaaaacgttaaacctcagcagtcgctcgacgaatgggctgcggttgggaagcccacgaggcctatagccagagcctcgagttgacaggagcccagacgccttttccaacggcaacttttatataaaatggcaatgtattcatgcaattgcggccgtgtcaggttggagacactggaccacactctccattgcttcctgaggagatggatcattgctagtgcatctacgcgcagcaatcccgcaagctcgacaaccgtagatgggctttggtgggccaatcaattacgcaacccgcacgttaaattgtatgaggaaggaaggccacggtacaaagtgggtggtcttcacccagtggttgttggtggcgtcatgcagaccatgcattggggatagcacagggttggggtgtcttgtggactcaatgggtgaaaggagatggaaaagggcggtgaaaagtggtagaatcgaaatccctgacgtcaatttataaagtaaaatgcgtttctgccattttgctcccctccttctttcgcaatcgcctccccaaaagttgtcgtggcagtacacatgcttgcatacaatgaagctaatccggcttgctcagtagttgctatatccaggcatggtgtgaaacccctcaaagtatatataggagcggtgagccccagtctggggtcttttctctccatctcaaaactactttctcacatgctagccacaaaaatgaccactaagtacacttccgttcacgagtctcccaacggccctggtgacgctcgacccaccgcttcccagattatcgacgattacaaccttgagggagagctttctggcaagactgttctcgtcaccggctgttcctctggtattggtgttgagactgcccgagctatttaccgaactggtgccaccctttacctcactgcccgagatgtcgataaggccaagaccgttcttcccgaccttgttgacacttcccgagtccactttctccaccttgaccttaactctctggagtctgttcgaggttttgctgagaacttcaagtctaagtccactcagcttcacattctcatcgagaacgctggcgtgatggcctgtcccgagggccgaaccgtcgatggttttgagactcagtttggtatcaaccaccttgctcactttctcctcttttacctcctcaaggatacccttctcaactcttctacccccgctttcaactcccgagttgtcatcctctcttcttgtgctcaccaggctggttccgttcaccttaacaacctgtctcttgagggtggatacgagccttggaagtcttacggccagtccaagactgccaacctttggactgcccgagagatcgagaagcgatttggtgcttccggtatccactcttgggctgttcaccccggttccatcgctactgagcttcagcgacacgtttccgacgagcttaagcagaagtgggctgacgataaggagggtgccaagctgtggaagtccaccgagcagggtgccgccaccactgtccttgctgctgtttcccctgagcttgagggtaagggcggtctttaccttgaggatacccaggttgccaagccccctgcccgaggaatgtttggtgttgctgactgggcttacgatgaggatggcccctctaagctctgggccaagtctcttgagctccttaagctccagtaaaggttagactatggatatgtaatttaactgtgtatatagagagcgtgcaagtatggagcgcttgttcagcttgtatgatggtcagacgacctgtctgatcgagtatgtatgatactgcacaacctgtgtatccgcatgatctgtccaatggggcatgttgttgtgtttctcgatacggagatgctgggtacaagtagctaatacgattgaactacttatacttatatgaggcttgaagaaagctgacttgtgtatgacttattctcaactacatccccagtcacaataccaccactgcactaccactacacactagtggtgtgttctgtggagcattctcacttttggtaaacgacattgcttcaagtgcagcggaatcaaaaagtataaagtgggcagcgagtatacctgtacagactgtaggcgataactcaatccaattaccccccacaacatgactggccaaactgatctcaagactttattgaaatcagcaacaccgattctcaatgaaggcacatacttcttctgcaacattcacttgacgcctaaagttggtgagaaatggaccgacaagacatattctgctatccacggactgttgcctgtgtcggtggctacaatacgtgagtcagaagggctgacggtggtggttcccaaggaaaaggtcgacgagtatctgtctgactcgtcattgccgcctttggagtacgactccaactatgagtgtgcttggatcactttgacgatacattcttcgttggaggctgtgggtctgacagctgcgttttcggcgcggttggccgacaacaatatcagctgcaacgtcattgctggctttcatcatgatcacatttttgtcggcaaaggcgacgcccagagagccattgacgttctttctaatttggaccgatagccgtatagtccagtctatctataagttcaactaactcgtaactattaccataacatatacttcactgccccagataaggttccgataaaaagttctgcagactaaatttatttcagtctcctcttcaccaccaaaatgccctcctacgaagctcgagctaacgtccacaagtccgcctttgccgctcgagtgctcaagctcgtggcagccaagaaaaccaacctgtgtgcttctctggatgttaccaccaccaaggagctcattgagcttgccgataaggtcggaccttatgtgtgcatgatcaagacccatatcgacatcattgacgacttcacctacgccggcactgtgctccccctcaaggaacttgctcttaagcacggtttcttcctgttcgaggacagaaagttcgcagatattggcaacactgtcaagcaccagtacaagaacggtgtctaccgaatcgccgagtggtccgatatcaccaacgcccacggtgtacccggaaccggaatcattgctggcctgcgagctggtgccgaggaaactgtctctgaacagaagaaggaggacgtctctgactacgagaactcccagtacaaggagttcctggtcccctctcccaacgagaagctggccagaggtctgctcatgctggccgagctgtcttgcaagggctctctggccactggcgagtactccaagcagaccattgagcttgcccgatccgaccccgagtttgtggttggcttcattgcccagaaccgacctaagggcgactctgaggactggcttattctgacccccggggtgggtcttgacgacaagggagacgctctcggacagcagtaccgaactgttgaggatgtcatgtctaccggaacggatatcataattgtcggccgaggtctgtacggccagaaccgagatcctattgaggaggccaagcgataccagaaggctggctgggaggcttaccagaagattaactgttagaggttagactatggatatgtaatttaactgtgtatatagagagcgtgcaagtatggagcgcttgttcagcttgtatgatggtcagacgacctgtctgatcgagtatgtatgatactgcacaacctgtgtatccgcatgatctgtccaatggggcatgttgttgtgtttctcgatacggagatgctgggtacaagtagctaatacgattgaactacttatacttatatgaggcttgaagaaagctgacttgtgtatgacttattctcaactacatccccagtcacaataccaccactgcactaccactacacctcgagcatgcacactattatcacattactacatccaaacccctacagggggaggagctctccaatcaaatatgtacattaactatctctcgtaaatcattgttataagaccgtccgtgactgtctaaatcggttcattcgttgtaacaaatcagtgtaacaactcgtggtacgcccggtttgcttcgctcacgctcccctagattttccgtctaggacacaacaagccctggtggatgacgttcaacgccttcagcgcgtctttttcctcaataacacacgagatgttaatttcgttggctccctgagaaatcatctcaatgttaatacctgcctgggccagagtagagaagaacatgcctgcacatccgaccatggccttcattctcgttccgatcagcgacacaatggtcatgcctcgcttcacatctactgtgccgtactttcgcagctcctccacagcctgcttgaggttggagtcgggagcatggaaggccatcgacacatggacctcagaagtggagatgagatcgacgacaagtttctgctggtcgagagtagcaaagatcttgttcaagaagccatgactcttggttcgcttattcgaatgaacgttgagaacggtgatattcgatttggtagtgacagctgtaggcttcttctcgtcatctacaggagcagacacctggggagtgaatgagccagaggacagagaagttagcgagtcggtggaagaagccagatcctggacattgtttttcgttttcaggttgcccgagccgtcagcagatgggtagatgatagttcctcctcccagggggttttccacgtttttgattcggataggaatatgggccttaatgacctgctccatggtgaaggggtggatgacttcagatccgtagtaggtcaactcagcggcctcctcgggggtaatgatgggcagcagacgggcagtggacacctttctgggatcggcagtgaagacaccatcgacttctttccagatctgaagctccttggcgtccagacccacagccaccagagcagcacacagatcggtgtatcctcgtccgatctggcttaggaggcctcccttgacggggccaaagaaaccggtcaacacgggcaccatgtttcccttgacaggagcagagtccgtgttaggagagccgggaagagtgatgatctcgcccagaacacgtccgaggtccgaatagaacttgggatcttcggcattggtggtggtaactgcgtgagacaggtcaaagtaccgtgcgttaacaccagcgtcccgcataactgcagtcatgtacatgcaactgagcttctccccaatggccatgatggagtcgagtgttcggggggagatctcagaaatgatttcagcagcagccaggattcgcaacagctggtcgcactcgccgttgatgtcggcattgaggttttcgagcagttcggggttcttgacgtcacgcttagcagctgcaagatggtcttctcggatagactcaatgatggggttgtaggcgtctgatccgagaagagcagagtcagcagcagcaataagacgggtggtggttccctcggccttggtggcctctagatggcctccttggccccattccagctgcattaatgaatcggccaacgcgcggggagaggcggtttgcgtattgggcgctcttccgcttcctcgctcactgactcgctgcgctcggtcgttcggctgcggcgagcggtatcagctcactcaaaggcggtaatacggttatccacagaatcaggggataacgcaggaaagaacatgtgagcaaaaggccagcaaaaggccaggaaccgtaaaaaggccgcgttgctggcgtttttccataggctccgcccccctgacgagcatcacaaaaatcgacgctcaagtcagaggtggcgaaacccgacaggactataaagataccaggcgtttccccctggaagctccctcgtgcgctctcctgttccgaccctgccgcttaccggatacctgtccgcctttctcccttcgggaagcgtggcgctttctcatagctcacgctgtaggtatctcagttcggtgtaggtcgttcgctccaagctgggctgtgtgcacgaaccccccgttcagcccgaccgctgcgccttatccggtaactatcgtcttgagtccaacccggtaagacacgacttatcgccactggcagcagccactggtaacaggattagcagagcgaggtatgtaggcggtgctacagagttcttgaagtggtggcctaactacggctacactagaagaacagtatttggtatctgcgctctgctgaagccagttaccttcggaaaaagagttggtagctcttgatccggcaaacaaaccaccgctggtagcggtggtttttttgtttgcaagcagcagattacgcgcagaaaaaaaggatctcaagaagatcctttgatcttttctacggggtctgacgctcagtggaacgaaaactcacgttaagggattttggtcatgagattatcaaaaaggatcttcacctagatccttttaaattaaaaatgaagttttaaatcaatctaaagtatatatgagtaaacttggtctgacagttaccaatgcttaatcagtgaggcacctatctcagcgatctgtctatttcgttcatccatagttgcctgactccccgtcgtgtagataactacgatacgggagggcttaccatctggccccagtgctgcaatgataccgcgagagccacgctcaccggctccagatttatcagcaataaaccagccagccggaagggccgagcgcagaagtggtcctgcaactttatccgcctccatccagtctattaattgttgccgggaagctagagtaagtagttcgccagttaatagtttgcgcaacgttgttgccattgctacaggcatcgtggtgtcacgctcgtcgtttggtatggcttcattcagctccggttcccaacgatcaaggcgagttacatgatcccccatgttgtgcaaaaaagcggttagctccttcggtcctccgatcgttgtcagaagtaagttggccgcagtgttatcactcatggttatggcagcactgcataattctcttactgtcatgccatccgtaagatgcttttctgtgactggtgagtactcaaccaagtcattctgagaatagtgtatgcggcgaccgagttgctcttgcccggcgtcaatacgggataataccgcgccacatagcagaactttaaaagtgctcatcattggaaaacgttcttcggggcgaaaactctcaaggatcttaccgctgttgagatccagttcgatgtaacccactcgtgcacccaactgatcttcagcatcttttactttcaccagcgtttctgggtgagcaaaaacaggaaggcaaaatgccgcaaaaaagggaataagggcgacacggaaatgttgaatactcatactcttcctttttcaatattattgaagcatttatcagggttattgtctcatgagcggatacatatttgaatgtatttagaaaaataaacaaataggggttccgcgcacatttccccgaaaagtgccacctgacgtctaagaaaccattattatcatgacattaacctataaaaataggcgtatcacgag

SEQ ID NO: 11 - DNA, 13802 bp, Artificial Sequence
  expression plasmid
ggttccgcttcctcgctcactgactcgctgcgctcggtcgttcggctgcggcgagcggtatcagctcactcaaaggcggtaatacggttatccacagaatcaggggataacgcaggaaagaacatgtgagcaaaaggccagcaaaaggccaggaaccgtaaaaaggccgcgttgctggcgtttttccataggctccgcccccctgacgagcatcacaaaaatcgacgctcaagtcagaggtggcgaaacccgacaggactataaagataccaggcgtttccccctggaagctccctcgtgcgctctcctgttccgaccctgccgcttaccggatacctgtccgcctttctcccttcgggaagcgtggcgctttctcatagctcacgctgtaggtatctcagttcggtgtaggtcgttcgctccaagctgggctgtgtgcacgaaccccccgttcagcccgaccgctgcgccttatccggtaactatcgtcttgagtccaacccggtaagacacgacttatcgccactggcagcagccactggtaacaggattagcagagcgaggtatgtaggcggtgctacagagttcttgaagtggtggcctaactacggctacactagaaggacagtatttggtatctgcgctctgctgaagccagttaccttcggaaaaagagttggtagctcttgatccggcaaacaaaccaccgctggtagcggtggtttttttgtttgcaagcagcagattacgcgcagaaaaaaaggatctcaagaagatcctttgatcttttctacggggtctgacgctcagtggaacgaaaactcacgttaagggattttggtcatgagattatcaaaaaggatcttcacctagatccttttaaattaaaaatgaagttttaaatcaatctaaagtatatatgagtaaacttggtctgacagttaccaatgcttaatcagtgaggcacctatctcagcgatctgtctatttcgttcatccatagttgcctgactccccgtcgtgtagataactacgatacgggagggcttaccatctggccccagtgctgcaatgataccgcgagacccacgctcaccggctccagatttatcagcaataaaccagccagccggaagggccgagcgcagaagtggtcctgcaactttatccgcctccatccagtctattaattgttgccgggaagctagagtaagtagttcgccagttaatagtttgcgcaacgttgttgccattgctgcaggcatcgtggtgtcacgctcgtcgtttggtatggcttcattcagctccggttcccaacgatcaaggcgagttacatgatcccccatgttgtgcaaaaaagcggttagctccttcggtcctccgatcgttgtcagaagtaagttggccgcagtgttatcactcatggttatggcagcactgcataattctcttactgtcatgccatccgtaagatgcttttctgtgactggtgagtactcaaccaagtcattctgagaatagtgtatgcggcgaccgagttgctcttgcccggcgtcaacacgggataataccgcgccacatagcagaactttaaaagtgctcatcattggaaaacgttcttcggggcgaaaactctcaaggatcttaccgctgttgagatccagttcgatgtaacccactcgtgcacccaactgatcttcagcatcttttactttcaccagcgtttctgggtgagcaaaaacaggaaggcaaaatgccgcaaaaaagggaataagggcgacacggaaatgttgaatactcatactcttcctttttcaatattattgaagcatttatcagggttattgtctcatgagcggatacatatttgaatgtatttagaaaaataaacaaataggggttccgcgcacatttccccgaaaagtgccacctgacgtctaagaaaccattattatcatgacattaacctataaaaataggcgtatcacgaggccctttcgtctggcctaggaagcgacttccaatcgctttgcatatccagtaccacacccacaggcgtttgtgctactctactgatagcaatagatgcgtcataattggttggcccgctgagcctccacaggatactattgcacataccctggtcatgtgcagatcagctcatttgtggagactctggagtaacttagacgacgcctggttcaattgccgcaatgtgcgcccacgcagataatgtattgaggggtggagcgcctcttggggacttgctgtacttgtacgggatattaaacgcactcagcaagaccatgacgtaaaacacacctactgtacgatacgtactgtaggtattgtactcgtacccggtactacaaatagtacgatactatacggagtgtatttgtaccttgatatacgactggcggagtgaagagaaggagttgaacaagaccagatggggatatcagccccagtgctttgtattacaagtacgagtacttaatagatactgtaaggctattgatacggatggcagtaagtcattgagtaagcaattgtggcccagcatctcccctacgtacttgtaccataccccatggagacaccaatggtctttcacgcacactgtcgtgtgctgtatcgcagaatcgggtgtccaaccaaatgccgttacccccacgtcacagccgatagacagatacaccatcaataccagcaggttgtatcatgcggttggctgaaggtaagctgattggtctaaaaactgtagctgtcctaattcaacgagcgctatttggggccaaccacctcggccaagcggcctttaatctgcgtgccccagaggcgtctaatgaggctctggccgccactgtaggagtgtttctctgtgcgcacacgcagttttgagtttgggcgactttccctttttcccaattgcgtacacacacagctccgagctaagcgctgtccttgaaccttctccctcttttccctctttttctcttccccttcccctcctccacattaaggccaaatcctgaattgcaccaactagtacaacgacaacaatggacaagaagtactccatcggtttggacattggtactaactctgtcggctgggccgtcatcaccgacgagtacaaggttccctccaagaagttcaaggtccttggcaacaccgaccgacactctatcaagaagaacctgatcggtgctctgctgttcgactctggcgagactgccgaggccacccgactgaagcgaaccgctcgacgccgatacacccgacgaaagaaccgaatctgttacctccaggagatcttcagcaacgagatggctaaggtcgacgactccttcttccaccgactcgaggagtctttcctggtcgaagaggataagaagcacgagcgacaccccatcttcggcaacattgttgatgaggttgcctaccatgagaagtaccccaccatctaccacctccgaaagaagctcgtcgactccactgacaaggctgacctccgactcatctaccttgctctcgcccacatgatcaagttccgaggtcacttcctcattgagggtgatctcaaccccgacaactccgacgttgacaagctgttcatccagctcgtccagacctacaaccagctctttgaggagaaccctatcaacgcttctggtgttgacgccaaggccattctctccgcccgactctctaagtcccgacgactcgagaacctcattgcccagctgcccggcgagaagaagaacggcctcttcggtaacctgattgctctctctcttggtctgacccccaacttcaagtccaactttgacctcgccgaggacgccaagctccagctgtccaaggacacctacgatgacgatctggacaacctcctggcccagatcggtgaccagtacgccgatctcttccttgccgccaagaacctctccgacgccatcctgctctccgacatcctccgagtcaacaccgagattaccaaggctcctctgtctgcctctatgatcaagcgatacgacgagcaccaccaggatctcactcttctcaaggctctcgtccgacagcagctccccgagaagtacaaggagattttctttgaccagtccaagaacggttacgctggctacattgacggtggtgcttcccaggaagagttttacaagttcatcaagcctattctggagaagatggacggtaccgaggagctgctcgtcaagctcaaccgagaggacctccttcgaaagcagcgaaccttcgataacggctccatcccccaccagatccacctgggtgagctccacgccattctccgaagacaagaggacttctaccccttcctaaaggataaccgagagaagatcgagaagattctcaccttccgaatcccctactacgtcggtcccctcgctcgaggtaactcccgatttgcttggatgacccgaaagtccgaggagactatcaccccctggaactttgaagaggtagtcgacaagggtgcctccgcccagtctttcattgagcggatgaccaacttcgataagaacctccccaacgagaaggtccttcccaagcactctctcctctacgagtacttcaccgtctacaacgagctgaccaaggtcaagtacgttaccgagggcatgcgaaagcccgctttcctctctggtgagcagaagaaggccattgtcgacctcctgttcaagactaaccgaaaagtcaccgtcaagcagctcaaggaagactacttcaagaagattgagtgcttcgactccgtcgagatttccggtgtcgaggaccgattcaacgcctccctcggcacctaccacgatcttctgaagatcatcaaggacaaggactttcttgataacgaggagaacgaggacattctcgaggacatcgtcctcaccctcacccttttcgaggatcgagagatgatcgaggagcgactcaagacctacgcccatctcttcgacgacaaggtcatgaagcaactcaagcgacgacgatacactggctggggccgactttcccgaaagctcatcaacggcatccgagacaagcagtctggcaagaccatcctggacttcctgaagtccgacggtttcgccaaccgaaacttcatgcagctcatccacgacgactctcttaccttcaaagaggatatccagaaggcccaggtttctggccagggcgactccctccacgagcacattgccaacctcgccggatcccccgccatcaaaaagggtatcctccagaccgtcaaggttgtcgacgaactcgtgaaggtcatgggccgacacaagcccgagaacatcgttatcgagatggcccgagagaaccagaccacccagaagggtcagaagaactcccgagagcgaatgaagcgaatcgaagagggtatcaaggagctcggttcccagattctcaaggagcaccccgtcgagaacacccagctccagaacgagaaactctacctgtactacctccagaatggccgagacatgtacgttgaccaggagctcgacatcaaccgactctccgactacgacgtcgaccacattgttcctcagtccttcctcaaggacgactccatcgacaacaaggttctgacccgatctgacaagaaccgaggtaagtccgacaacgttccctccgaagaggtcgttaagaagatgaagaactactggcgacagcttctcaacgccaaactgatcacccagcgaaagtttgacaacctcaccaaggccgagcgaggtggtctgtccgagctggacaaggccggcttcattaagcgacagctggtcgagactcgacagatcaccaagcacgtcgcccagatcctcgactcccgaatgaacaccaagtacgacgagaacgacaagctcatccgggaggtcaaggtcatcaccctgaagtctaagcttgtctccgacttccgaaaggacttccagttctacaaggtccgagagatcaacaactaccaccacgcccacgacgcctacctcaacgccgttgttggtaccgccctcatcaagaagtatcccaagctcgagtccgagttcgtttacggcgactacaaggtttacgatgtccgaaagatgattgccaagtccgagcaggagatcggtaaggccaccgccaagtactttttctactccaacatcatgaatttcttcaagaccgagatcactctcgccaacggtgagattcgaaagcgacccctgattgagactaatggtgagactggtgagatcgtctgggataagggccgagacttcgccaccgtccgaaaggtcctgtccatgccccaggtcaacattgtcaagaagaccgaggtccagaccggtggcttctccaaggagtccattctccccaagcgaaactccgacaaactcatcgcccgtaagaaggactgggatccgaagaagtacggtggtttcgattctcccaccgttgcctactccgtcctcgttgttgctaaagtcgagaagggtaagtctaagaaactcaagtccgtgaaggagctactcggtatcaccatcatggagcgatcttcttttgagaagaaccccattgacttcctcgaggccaagggttacaaagaggtcaagaaggacctgattatcaagctgcccaagtactccctctttgagctcgagaacggccgaaagcgaatgctggcttccgctggtgagctgcagaagggcaacgagctcgctctgccctccaagtacgtcaacttcctctacctggcctcccactacgagaagctcaagggctcccccgaggacaacgagcagaagcagctgttcgttgagcagcacaagcactacctcgacgagatcatcgagcagatctccgagttctccaagcgagtcatcctcgctgacgccaaccttgataaggttctctctgcttacaacaagcaccgggacaagcccatccgagagcaggccgagaatatcatccacctcttcactctcaccaacctcggcgctcctgctgccttcaagtacttcgacaccaccattgaccgaaagaggtacacctccaccaaggaagtcctcgacgccaccctgatccaccagtccatcaccggcctctacgaaacccgaatcgacctctcccagctcggcggtgactctcgagccgaccccaagaagaagcgaaaagtctaaatatccgaagatcaagagcgaagcaagttgtaagtccaggacatgtttcccgcccacgcgagtgatttataacacctctcttttttgacacccgctcgccttgaaattcatgtcacataaattatagtcaacgacgtttgaataacttgtcttgtagttcgatgatgatcatatgattacattaatagtaattactgtatttgatatatatactaattacaatagtacatattagaacatacaatagttagtgccgtgaagtggcttaaaataccgcgagtcgattacgtaatattattacctcttgcccatcgaacgtacaagtactcctctgttctctccttcctttgctttgtgcacgaagaactgcggtcaggtgacacaactttttccatctcagggtgtgtcgcgtgtgcttcatccaaactttagttggggttcgggttcgcgcgagatgatcacgtgccctgatttggtgtcgtcccccgtcgcgctgcgcacgtgatttatttatttccggtggctgctgtctacgcggggccttctctgcccttctgtttcaaccttcgggcggttctcgtaaccagcagtagcaatccatttcgaaactcaaagagctaaaaacgttaaacctcagcagtcgctcgacgaatgggctgcggttgggaagcccacgaggcctatagccagagcctcgagttgacaggagcccagacgccttttccaacggcaacttttatataaaatggcaatgtattcatgcaattgcggccgtgtcaggttggagacactggaccacactctccattgcttcctgaggagatggatcattgctagtgcatctacgcgcagcaatcccgcaagctcgacaaccgtagatgggctttggtgggccaatcaattacgcaacccgcacgttaaattgtatgaggaaggaaggccacggtacaaagtgggtggtcttcacccagtggttgttggtggcgtcatgcagaccatgcattggggatagcacagggttggggtgtcttgtggactcaatgggtgaaaggagatggaaaagggcggtgaaaagtggtagaatcgaaatccctgacgtcaatttataaagtaaaatgcgtttctgccattttgctcccctccttctttcgcaatcgcctccccaaaagttgtcgtggcagtacacatgcttgcatacaatgaagctaatccggcttgctcagtagttgctatatccaggcatggtgtgaaacccctcaaagtatatataggagcggtgagccccagtctggggtcttttctctccatctcaaaactactttctcacaatggatttgctgatgagtccgtgaggacgaaacgagtaagctcgtctggaggcatgatcaacagcggttttagagctagaaatagcaagttaaaataaggctagtccgttatcaacttgaaaaagtggcaccgagtcggtgcttttggccggcatggtcccagcctcctcgctggcgccggctgggcaacatgcttcggcatggcgaatgggactaaacttcgagctaatccagtagcttacgttacccaggggcaggtcaactggctagccacgagtctgtcccaggtcgcaatttagtgtaataaacaatatatatattgagtctaaagggaattgtagctattgtgattgtgtgattttcgtcttgctggttcttattgtgtcccattcgtttcatcctgatgaggacccctggaaccggtgttttcttagtctctgcaatcgctagtcttgttgctatgacagttgcgtcgacactattcaggtcatctatcggttattctgatattataatacctccggatcgatgtacctgatttatacttgcagcaatgtttacttcttatcgttggaccccgtcttcaattacacttcccaactgggaacacccctctttatcgacccattttaggtaatttaccctagcccattgtctccataaggaatattaccctaacccacagtccagggtgcccaggtccttctttggccaaattttaacttcggtcctatggcacagcggtagcgcgtgagattgcaaatcttaaggtcccgagttcgaatctcggtgggacctagttgaaaaatacctctaatgcgccgatggtttagtggtaaaatccatcgttgccatcgatgggcccccggttcgattccgggtcggcgcaggttgacgtacagcaggctgaacgaggatgttttagagctagaaatagcaagttaaaataaggctagtccgttatcaacttgaaaaagtggcaccgagtcggtgcttttttttttcgatcggccccagttgcaaaagttgacacaactctagatctgcttccaaatatagaatcataacaagggttagggtgtgattatataatattggtcttaattgatgtgctagggctttaaaagttggttaaaataacgctctaatgcctttttaatatattgtctttttcaaaatctcaaatcggacacttcttcgtgtatgagactccattttttggctccgtcacgtgatatgtattatcagctatagtggtgtaaacaaagttttttactagctgtaatggcattttgtcggagtggtaaatcgccttcttgttgtgcgttcgagttctggactctgcactgggctactttgaaaaatacctctaatgcgccgatggtttagtggtaaaatccatcgttgccatcgatgggcccccggttcgattccgggtcggcgcaggttgacgttcactcctcagcctcccaaggttttagagctagaaatagcaagttaaaataaggctagtccgttatcaacttgaaaaagtggcaccgagtcggtgcttttttttttcgcgatacacgaatgtgatacggatcaaagtaagcaggactacgataagataacgaatgcggtgcagtccatgtcgattaggtatagatacatttattttgtgttatgttacattttggggggatactgtcctacttgtagtacctacttgtagtggcgcgtctattcctttgccctcggacgagtgctggggcgtcggtttccactatcggcgagtacttctacacagccatcggtccagacggccgcgcttctgcgggcgatttgtgtacgcccgacagtcccggctccggatcggacgattgcgtcgcatcgaccctgcgcccaagctgcatcatcgaaattgccgtcaaccaagctctgatagagttggtcaagaccaatgcggagcatatacgcccggagccgcggcgatcctgcaagctccggatgcctccgctcgaagtagcgcgtctgctgctccatacaagccaaccacggcctccagaagaagatgttggcgacctcgtattgggaatccccgaacatcgcctcgctccagtcaatgaccgctgttatgcggccattgtccgtcaggacattgttggagccgaaatccgcgtgcacgaggtgccggacttcggggcagtcctcggcccaaagcatcagctcatcgagagcctgcgcgacggacgcactgacggtgtcgtccatcacagtttgccagtgatacacatggggatcagcaatcgcgcatatgaaatcacgccatgtagtgtattgaccgattccttgcggtccgaatgggccgaacccgctcgtctggctaagatcggccgcagcgatcgcatccatggcctccgcgaccggctgcagaacagcgggcagttcggtttcaggcaggtcttgcaacgtgacaccctgtgcacggcgggagatgcaataggtcaggctctcgctgaattccccaatgtcaagcacttccggaatcgggagcgcggccgatgcaaagtgccgataaacataacgatctttgtagaaaccatcggcgcagctatttacccgcaggacatatccacgccctcctacatcgaagctgaaagcacgagattcttcgccctccgagagctgcatcaggtcggagacgctgtcgaacttttcgatcagaaacttctcgacagacgtcgcggtgagttcaggctttttcatatgggtacctgagaacatttttgtgtctaggtgtttgtgtttggactgcgatcagtgaagaaaagaagaggaaaaattgtgcaagaaattttgctttcaagacttggctgatgcagcagggtaactctgggacacagacctatgtttgtggttaaactcaatgcacgtggtacgtgcgtggagcgcttacccatccaagggtgtggacatggaaccgacggtccgtggagttgtgtaatgtcattttggcgactcttgaagcaaggctataaaaaaattgtgtggcttgagtcttatcgagctcggtcactacaagagttaatcttcctgtctcaggcagacaggtcaggcagggttacttttgggtgtgctgtaactcactgtatggccgttagtgcgcatagacgttgtacatactggaccgaattgtagcgtgctcaatagggccaataaagctattgtagggatccgaattttcagaacctaatttatctgttacccggcctgtggctcgcacagcttaaaaatggtcaaactttccccttcttgtctttttttcctcacattcatcaggttcttgtcttgatctttcaagtgagtattaattaccgaccttggttcttcattgggagagcattggaagccgtggtgcagcaaccacaaaacggttcttccccttcgataccttcttgcctgcctttcaatacaagtcggctcgattagcggtggtcgcccccgccagcggagaacatggaactaacccagaatgagagctaagtggagaaagaagagagtcagacgactcaagcgaaagcgccgcaaggtccgagctcgatccaaataagcggtttttaacggagatttaacactaaatcgaagaacttttcccgtttcatttgcgaatgagctcgttaacaaaatcccccagtttttttatccagctgtaaggattgacattagtaatgaattattgtttggtatatttaaatctgtagttcctttctgtccgtgtcggcaactgtcgtactcgtgatttacttgtattgacgaatacttactgtagcgcactctgctgctactggtcgtaaggatgtgctatttcggtgtatggtgggttttttgggggtcggaaccgaagactgttacacgggcacggctcgttgtgtacacgcacagagctcttgcgagtcatgttgtagctagctcgtcgtgttcaggaactgttcgatggttcggagagagtcgccgcccagaacatacgcgcaccgatgtcagcagacagccttattacaagtatattcaagcaagtatatccgtagggtgcgggtgatttggatctaaggttcgtactcaacactcacgagcagcttgcctatgttacatccttttatcagacataacataattggagtttacttacacacggggtgtacctgtatgagcaccacctacaattgtagcactggtacttgtacaaagaatttattcgtacgaatcacagggacggccgccctcaccgaaccagcgaatacctcagcggtcccctgcagtgactcaacaaagcgatatgaacatcttgcgatggtatcctgctgatagtttttactgtacaaacacctgtgtagctccttctagcatttttaagttattcacacctcaaggggagggataaattaaataaattccaaaagcgaagatcgagaaactaaattaaaattccaaaaacgaagttggaacacaaccccccgaaaaaaaacaacaaacaaaaaacccaacaaaataaacaaaaacaaaataaatatataactaccagtatctgactaaaagttcaaatactcgtacttacaacaaatagaaatgagccggccaaaattctgcagaaaaaaatttcaaacaagtactggtataattaaattaaaaaacacatcaaagtatcataacgttagttattttattttatttaataaaagaaaacaacaagatgggctcaaaactttcaacttatacgatacataccaaataacaatttagtatttatctaagtgcttttcgtagataatggaatacaaatggatatccagagtatacacatggatagtatacactgacacgacaattctgtatctctttatgttaactactgtgaggcattaaatagagcttgatatataaaatgttacatttcacagtctgaacttttgcagattacctaatttggtaagatattaattatgaactgaaagttgatggcatccctaaatttgatgaaagatgaaattgtaaatgaggtggtaaaagagctacagtcgttttgttttgagataccatcatctctaacgaaatatctattaaaaatctcagtgtgatcatgagtcattgccatcctggaaaatgtcatcatggctgatatttctaactgtttacttgagataaatatatatttacaagaacttcccttgaaattaatttagatataaaatgtttgcgggcaagttactacgaggaataaattatatctaga

SEQ ID NO: 12 - DNA, 13246 bp, Artificial Sequence
  expression plasmid
ggttccgcttcctcgctcactgactcgctgcgctcggtcgttcggctgcggcgagcggtatcagctcactcaaaggcggtaatacggttatccacagaatcaggggataacgcaggaaagaacatgtgagcaaaaggccagcaaaaggccaggaaccgtaaaaaggccgcgttgctggcgtttttccataggctccgcccccctgacgagcatcacaaaaatcgacgctcaagtcagaggtggcgaaacccgacaggactataaagataccaggcgtttccccctggaagctccctcgtgcgctctcctgttccgaccctgccgcttaccggatacctgtccgcctttctcccttcgggaagcgtggcgctttctcatagctcacgctgtaggtatctcagttcggtgtaggtcgttcgctccaagctgggctgtgtgcacgaaccccccgttcagcccgaccgctgcgccttatccggtaactatcgtcttgagtccaacccggtaagacacgacttatcgccactggcagcagccactggtaacaggattagcagagcgaggtatgtaggcggtgctacagagttcttgaagtggtggcctaactacggctacactagaaggacagtatttggtatctgcgctctgctgaagccagttaccttcggaaaaagagttggtagctcttgatccggcaaacaaaccaccgctggtagcggtggtttttttgtttgcaagcagcagattacgcgcagaaaaaaaggatctcaagaagatcctttgatcttttctacggggtctgacgctcagtggaacgaaaactcacgttaagggattttggtcatgagattatcaaaaaggatcttcacctagatccttttaaattaaaaatgaagttttaaatcaatctaaagtatatatgagtaaacttggtctgacagttaccaatgcttaatcagtgaggcacctatctcagcgatctgtctatttcgttcatccatagttgcctgactccccgtcgtgtagataactacgatacgggagggcttaccatctggccccagtgctgcaatgataccgcgagacccacgctcaccggctccagatttatcagcaataaaccagccagccggaagggccgagcgcagaagtggtcctgcaactttatccgcctccatccagtctattaattgttgccgggaagctagagtaagtagttcgccagttaatagtttgcgcaacgttgttgccattgctgcaggcatcgtggtgtcacgctcgtcgtttggtatggcttcattcagctccggttcccaacgatcaaggcgagttacatgatcccccatgttgtgcaaaaaagcggttagctccttcggtcctccgatcgttgtcagaagtaagttggccgcagtgttatcactcatggttatggcagcactgcataattctcttactgtcatgccatccgtaagatgcttttctgtgactggtgagtactcaaccaagtcattctgagaatagtgtatgcggcgaccgagttgctcttgcccggcgtcaacacgggataataccgcgccacatagcagaactttaaaagtgctcatcattggaaaacgttcttcggggcgaaaactctcaaggatcttaccgctgttgagatccagttcgatgtaacccactcgtgcacccaactgatcttcagcatcttttactttcaccagcgtttctgggtgagcaaaaacaggaaggcaaaatgccgcaaaaaagggaataagggcgacacggaaatgttgaatactcatactcttcctttttcaatattattgaagcatttatcagggttattgtctcatgagcggatacatatttgaatgtatttagaaaaataaacaaataggggttccgcgcacatttccccgaaaagtgccacctgacgtctaagaaaccattattatcatgacattaacctataaaaataggcgtatcacgaggccctttcgtctggcctaggaagcgacttccaatcgctttgcatatccagtaccacacccacaggcgtttgtgctactctactgatagcaatagatgcgtcataattggttggcccgctgagcctccacaggatactattgcacataccctggtcatgtgcagatcagctcatttgtggagactctggagtaacttagacgacgcctggttcaattgccgcaatgtgcgcccacgcagataatgtattgaggggtggagcgcctcttggggacttgctgtacttgtacgggatattaaacgcactcagcaagaccatgacgtaaaacacacctactgtacgatacgtactgtaggtattgtactcgtacccggtactacaaatagtacgatactatacggagtgtatttgtaccttgatatacgactggcggagtgaagagaaggagttgaacaagaccagatggggatatcagccccagtgctttgtattacaagtacgagtacttaatagatactgtaaggctattgatacggatggcagtaagtcattgagtaagcaattgtggcccagcatctcccctacgtacttgtaccataccccatggagacaccaatggtctttcacgcacactgtcgtgtgctgtatcgcagaatcgggtgtccaaccaaatgccgttacccccacgtcacagccgatagacagatacaccatcaataccagcaggttgtatcatgcggttggctgaaggtaagctgattggtctaaaaactgtagctgtcctaattcaacgagcgctatttggggccaaccacctcggccaagcggcctttaatctgcgtgccccagaggcgtctaatgaggctctggccgccactgtaggagtgtttctctgtgcgcacacgcagttttgagtttgggcgactttccctttttcccaattgcgtacacacacagctccgagctaagcgctgtccttgaaccttctccctcttttccctctttttctcttccccttcccctcctccacattaaggccaaatcctgaattgcaccaactagtacaacgacaacaatggacaagaagtactccatcggtttggacattggtactaactctgtcggctgggccgtcatcaccgacgagtacaaggttccctccaagaagttcaaggtccttggcaacaccgaccgacactctatcaagaagaacctgatcggtgctctgctgttcgactctggcgagactgccgaggccacccgactgaagcgaaccgctcgacgccgatacacccgacgaaagaaccgaatctgttacctccaggagatcttcagcaacgagatggctaaggtcgacgactccttcttccaccgactcgaggagtctttcctggtcgaagaggataagaagcacgagcgacaccccatcttcggcaacattgttgatgaggttgcctaccatgagaagtaccccaccatctaccacctccgaaagaagctcgtcgactccactgacaaggctgacctccgactcatctaccttgctctcgcccacatgatcaagttccgaggtcacttcctcattgagggtgatctcaaccccgacaactccgacgttgacaagctgttcatccagctcgtccagacctacaaccagctctttgaggagaaccctatcaacgcttctggtgttgacgccaaggccattctctccgcccgactctctaagtcccgacgactcgagaacctcattgcccagctgcccggcgagaagaagaacggcctcttcggtaacctgattgctctctctcttggtctgacccccaacttcaagtccaactttgacctcgccgaggacgccaagctccagctgtccaaggacacctacgatgacgatctggacaacctcctggcccagatcggtgaccagtacgccgatctcttccttgccgccaagaacctctccgacgccatcctgctctccgacatcctccgagtcaacaccgagattaccaaggctcctctgtctgcctctatgatcaagcgatacgacgagcaccaccaggatctcactcttctcaaggctctcgtccgacagcagctccccgagaagtacaaggagattttctttgaccagtccaagaacggttacgctggctacattgacggtggtgcttcccaggaagagttttacaagttcatcaagcctattctggagaagatggacggtaccgaggagctgctcgtcaagctcaaccgagaggacctccttcgaaagcagcgaaccttcgataacggctccatcccccaccagatccacctgggtgagctccacgccattctccgaagacaagaggacttctaccccttcctaaaggataaccgagagaagatcgagaagattctcaccttccgaatcccctactacgtcggtcccctcgctcgaggtaactcccgatttgcttggatgacccgaaagtccgaggagactatcaccccctggaactttgaagaggtagtcgacaagggtgcctccgcccagtctttcattgagcggatgaccaacttcgataagaacctccccaacgagaaggtccttcccaagcactctctcctctacgagtacttcaccgtctacaacgagctgaccaaggtcaagtacgttaccgagggcatgcgaaagcccgctttcctctctggtgagcagaagaaggccattgtcgacctcctgttcaagactaaccgaaaagtcaccgtcaagcagctcaaggaagactacttcaagaagattgagtgcttcgactccgtcgagatttccggtgtcgaggaccgattcaacgcctccctcggcacctaccacgatcttctgaagatcatcaaggacaaggactttcttgataacgaggagaacgaggacattctcgaggacatcgtcctcaccctcacccttttcgaggatcgagagatgatcgaggagcgactcaagacctacgcccatctcttcgacgacaaggtcatgaagcaactcaagcgacgacgatacactggctggggccgactttcccgaaagctcatcaacggcatccgagacaagcagtctggcaagaccatcctggacttcctgaagtccgacggtttcgccaaccgaaacttcatgcagctcatccacgacgactctcttaccttcaaagaggatatccagaaggcccaggtttctggccagggcgactccctccacgagcacattgccaacctcgccggatcccccgccatcaaaaagggtatcctccagaccgtcaaggttgtcgacgaactcgtgaaggtcatgggccgacacaagcccgagaacatcgttatcgagatggcccgagagaaccagaccacccagaagggtcagaagaactcccgagagcgaatgaagcgaatcgaagagggtatcaaggagctcggttcccagattctcaaggagcaccccgtcgagaacacccagctccagaacgagaaactctacctgtactacctccagaatggccgagacatgtacgttgaccaggagctcgacatcaaccgactctccgactacgacgtcgaccacattgttcctcagtccttcctcaaggacgactccatcgacaacaaggttctgacccgatctgacaagaaccgaggtaagtccgacaacgttccctccgaagaggtcgttaagaagatgaagaactactggcgacagcttctcaacgccaaactgatcacccagcgaaagtttgacaacctcaccaaggccgagcgaggtggtctgtccgagctggacaaggccggcttcattaagcgacagctggtcgagactcgacagatcaccaagcacgtcgcccagatcctcgactcccgaatgaacaccaagtacgacgagaacgacaagctcatccgggaggtcaaggtcatcaccctgaagtctaagcttgtctccgacttccgaaaggacttccagttctacaaggtccgagagatcaacaactaccaccacgcccacgacgcctacctcaacgccgttgttggtaccgccctcatcaagaagtatcccaagctcgagtccgagttcgtttacggcgactacaaggtttacgatgtccgaaagatgattgccaagtccgagcaggagatcggtaaggccaccgccaagtactttttctactccaacatcatgaatttcttcaagaccgagatcactctcgccaacggtgagattcgaaagcgacccctgattgagactaatggtgagactggtgagatcgtctgggataagggccgagacttcgccaccgtccgaaaggtcctgtccatgccccaggtcaacattgtcaagaagaccgaggtccagaccggtggcttctccaaggagtccattctccccaagcgaaactccgacaaactcatcgcccgtaagaaggactgggatccgaagaagtacggtggtttcgattctcccaccgttgcctactccgtcctcgttgttgctaaagtcgagaagggtaagtctaagaaactcaagtccgtgaaggagctactcggtatcaccatcatggagcgatcttcttttgagaagaaccccattgacttcctcgaggccaagggttacaaagaggtcaagaaggacctgattatcaagctgcccaagtactccctctttgagctcgagaacggccgaaagcgaatgctggcttccgctggtgagctgcagaagggcaacgagctcgctctgccctccaagtacgtcaacttcctctacctggcctcccactacgagaagctcaagggctcccccgaggacaacgagcagaagcagctgttcgttgagcagcacaagcactacctcgacgagatcatcgagcagatctccgagttctccaagcgagtcatcctcgctgacgccaaccttgataaggttctctctgcttacaacaagcaccgggacaagcccatccgagagcaggccgagaatatcatccacctcttcactctcaccaacctcggcgctcctgctgccttcaagtacttcgacaccaccattgaccgaaagaggtacacctccaccaaggaagtcctcgacgccaccctgatccaccagtccatcaccggcctctacgaaacccgaatcgacctctcccagctcggcggtgactctcgagccgaccccaagaagaagcgaaaagtctaaatatccgaagatcaagagcgaagcaagttgtaagtccaggacatgtttcccgcccacgcgagtgatttataacacctctcttttttgacacccgctcgccttgaaattcatgtcacataaattatagtcaacgacgtttgaataacttgtcttgtagttcgatgatgatcatatgattacattaatagtaattactgtatttgatatatatactaattacaatagtacatattagaacatacaatagttagtgccgtgaagtggcttaaaataccgcgagtcgattacgtaatattattacctcttgcccatcgaacgtacaagtactcctctgttctctccttcctttgctttgtgcacgaagaactgcggtcaggtgacacaactttttccatctcagggtgtgtcgcgtgtgcttcatccaaactttagttggggttcgggttcgcgcgagatgatcacgtgccctgatttggtgtcgtcccccgtcgcgctgcgcacgtgatttatttatttccggtggctgctgtctacgcggggccttctctgcccttctgtttcaaccttcgggcggttctcgtaaccagcagtagcaatccatttcgaaactcaaagagctaaaaacgttaaacctcagcagtcgctcgacgaatgggctgcggttgggaagcccacgaggcctatagccagagcctcgagttgacaggagcccagacgccttttccaacggcaacttttatataaaatggcaatgtattcatgcaattgcggccgtgtcaggttggagacactggaccacactctccattgcttcctgaggagatggatcattgctagtgcatctacgcgcagcaatcccgcaagctcgacaaccgtagatgggctttggtgggccaatcaattacgcaacccgcacgttaaattgtatgaggaaggaaggccacggtacaaagtgggtggtcttcacccagtggttgttggtggcgtcatgcagaccatgcattggggatagcacagggttggggtgtcttgtggactcaatgggtgaaaggagatggaaaagggcggtgaaaagtggtagaatcgaaatccctgacgtcaatttataaagtaaaatgcgtttctgccattttgctcccctccttctttcgcaatcgcctccccaaaagttgtcgtggcagtacacatgcttgcatacaatgaagctaatccggcttgctcagtagttgctatatccaggcatggtgtgaaacccctcaaagtatatataggagcggtgagccccagtctggggtcttttctctccatctcaaaactactttctcacaatgacgagactgatgagtccgtgaggacgaaacgagtaagctcgtcggtggcctggattcgagtgggttttagagctagaaatagcaagttaaaataaggctagtccgttatcaacttgaaaaagtggcaccgagtcggtgcttttggccggcatggtcccagcctcctcgctggcgccggctgggcaacatgcttcggcatggcgaatgggactaaacttcgagctaatccagtagcttacgttacccaggggcaggtcaactggctagccacgagtctgtcccaggtcgcaatttagtgtaataaacaatatatatattgagtctaaagggaattgtagctattgtgattgtgtgattttcgtcttgctggttcttattgtgtcccattcgtttcatcctgatgaggacccctggaaccggtgttttcttagtctctgcaatcgctagtcttgttgctatgacagttgcgtcgacactattcaggtcatctatcggttattctgatattataatacctccggatcgatgtacctgatttatacttgcagcaatgtttacttcttatcgttggaccccgtcttcaattacacttcccaactgggaacacccctctttatcgacccattttaggtaatttaccctagcccattgtctccataaggaatattaccctaacccacagtccagggtgcccaggtccttctttggccaaattttaacttcggtcctatggcacagcggtagcgcgtgagattgcaaatcttaaggtcccgagttcgaatctcggtgggacctagttgaaaaatacctctaatgcgccgatggtttagtggtaaaatccatcgttgccatcgatgggcccccggttcgattccgggtcggcgcaggttgacgtttacacccactctatcggaggttttagagctagaaatagcaagttaaaataaggctagtccgttatcaacttgaaaaagtggcaccgagtcggtgcttttttttttcgcgatacacgaatgtgatacggatcaaagtaagcaggactacgataagataacgaatgcggtgcagtccatgtcgattaggtatagatacatttattttgtgttatgttacattttggggggatactgtcctacttgtagtacctacttgtagtggcgcgtctattcctttgccctcggacgagtgctggggcgtcggtttccactatcggcgagtacttctacacagccatcggtccagacggccgcgcttctgcgggcgatttgtgtacgcccgacagtcccggctccggatcggacgattgcgtcgcatcgaccctgcgcccaagctgcatcatcgaaattgccgtcaaccaagctctgatagagttggtcaagaccaatgcggagcatatacgcccggagccgcggcgatcctgcaagctccggatgcctccgctcgaagtagcgcgtctgctgctccatacaagccaaccacggcctccagaagaagatgttggcgacctcgtattgggaatccccgaacatcgcctcgctccagtcaatgaccgctgttatgcggccattgtccgtcaggacattgttggagccgaaatccgcgtgcacgaggtgccggacttcggggcagtcctcggcccaaagcatcagctcatcgagagcctgcgcgacggacgcactgacggtgtcgtccatcacagtttgccagtgatacacatggggatcagcaatcgcgcatatgaaatcacgccatgtagtgtattgaccgattccttgcggtccgaatgggccgaacccgctcgtctggctaagatcggccgcagcgatcgcatccatggcctccgcgaccggctgcagaacagcgggcagttcggtttcaggcaggtcttgcaacgtgacaccctgtgcacggcgggagatgcaataggtcaggctctcgctgaattccccaatgtcaagcacttccggaatcgggagcgcggccgatgcaaagtgccgataaacataacgatctttgtagaaaccatcggcgcagctatttacccgcaggacatatccacgccctcctacatcgaagctgaaagcacgagattcttcgccctccgagagctgcatcaggtcggagacgctgtcgaacttttcgatcagaaacttctcgacagacgtcgcggtgagttcaggctttttcatatgggtacctgagaacatttttgtgtctaggtgtttgtgtttggactgcgatcagtgaagaaaagaagaggaaaaattgtgcaagaaattttgctttcaagacttggctgatgcagcagggtaactctgggacacagacctatgtttgtggttaaactcaatgcacgtggtacgtgcgtggagcgcttacccatccaagggtgtggacatggaaccgacggtccgtggagttgtgtaatgtcattttggcgactcttgaagcaaggctataaaaaaattgtgtggcttgagtcttatcgagctcggtcactacaagagttaatcttcctgtctcaggcagacaggtcaggcagggttacttttgggtgtgctgtaactcactgtatggccgttagtgcgcatagacgttgtacatactggaccgaattgtagcgtgctcaatagggccaataaagctattgtagggatccgaattttcagaacctaatttatctgttacccggcctgtggctcgcacagcttaaaaatggtcaaactttccccttcttgtctttttttcctcacattcatcaggttcttgtcttgatctttcaagtgagtattaattaccgaccttggttcttcattgggagagcattggaagccgtggtgcagcaaccacaaaacggttcttccccttcgataccttcttgcctgcctttcaatacaagtcggctcgattagcggtggtcgcccccgccagcggagaacatggaactaacccagaatgagagctaagtggagaaagaagagagtcagacgactcaagcgaaagcgccgcaaggtccgagctcgatccaaataagcggtttttaacggagatttaacactaaatcgaagaacttttcccgtttcatttgcgaatgagctcgttaacaaaatcccccagtttttttatccagctgtaaggattgacattagtaatgaattattgtttggtatatttaaatctgtagttcctttctgtccgtgtcggcaactgtcgtactcgtgatttacttgtattgacgaatacttactgtagcgcactctgctgctactggtcgtaaggatgtgctatttcggtgtatggtgggttttttgggggtcggaaccgaagactgttacacgggcacggctcgttgtgtacacgcacagagctcttgcgagtcatgttgtagctagctcgtcgtgttcaggaactgttcgatggttcggagagagtcgccgcccagaacatacgcgcaccgatgtcagcagacagccttattacaagtatattcaagcaagtatatccgtagggtgcgggtgatttggatctaaggttcgtactcaacactcacgagcagcttgcctatgttacatccttttatcagacataacataattggagtttacttacacacggggtgtacctgtatgagcaccacctacaattgtagcactggtacttgtacaaagaatttattcgtacgaatcacagggacggccgccctcaccgaaccagcgaatacctcagcggtcccctgcagtgactcaacaaagcgatatgaacatcttgcgatggtatcctgctgatagtttttactgtacaaacacctgtgtagctccttctagcatttttaagttattcacacctcaaggggagggataaattaaataaattccaaaagcgaagatcgagaaactaaattaaaattccaaaaacgaagttggaacacaaccccccgaaaaaaaacaacaaacaaaaaacccaacaaaataaacaaaaacaaaataaatatataactaccagtatctgactaaaagttcaaatactcgtacttacaacaaatagaaatgagccggccaaaattctgcagaaaaaaatttcaaacaagtactggtataattaaattaaaaaacacatcaaagtatcataacgttagttattttattttatttaataaaagaaaacaacaagatgggctcaaaactttcaacttatacgatacataccaaataacaatttagtatttatctaagtgcttttcgtagataatggaatacaaatggatatccagagtatacacatggatagtatacactgacacgacaattctgtatctctttatgttaactactgtgaggcattaaatagagcttgatatataaaatgttacatttcacagtctgaacttttgcagattacctaatttggtaagatattaattatgaactgaaagttgatggcatccctaaatttgatgaaagatgaaattgtaaatgaggtggtaaaagagctacagtcgttttgttttgagataccatcatctctaacgaaatatctattaaaaatctcagtgtgatcatgagtcattgccatcctggaaaatgtcatcatggctgatatttctaactgtttacttgagataaatatatatttacaagaacttcccttgaaattaatttagatataaaatgtttgcgggcaagttactacgaggaataaattatatctaga

SEQ ID NO: 13 - DNA, 20 bp, Artificial Sequence
  sequence used for Cas9 CRISPR targeting
acagcaggctgaacgaggat

SEQ ID NO: 14 - DNA, 20 bp, Artificial Sequence
  sequence used for Cas9 CRISPR targeting
tggaggcatgatcaacagcg

SEQ ID NO: 15 - DNA, 20 bp, Artificial Sequence
  sequence used for Cas9 CRISPR targeting
tcactcctcagcctcccaag

SEQ ID NO: 16 - DNA, 20 bp, Artificial Sequence
  sequence used for Cas9 CRISPR targeting
ggtggcctggattcgagtgg

SEQ ID NO: 17 - DNA, 20 bp, Artificial Sequence
  sequence used for Cas9 CRISPR targeting
ttacacccactctatcggag